European Patent Specification EP 3 703 710 B9, published December 4, 2024. Title: METHODS AND COMPOSITIONS FOR DOSING OF ALLOGENEIC CHIMERIC ANTIGEN RECEPTOR T CELLS. Applicant: ALLOGENE THERAPEUTICS, INC. LES LABORATOIRES SERVIER. The sequence listing filed with the application follows.

SEQUENCE LISTING (35 sequences)

SEQ ID NO: 1 - protein, 495 aa, Artificial Sequence
  CAR full length amino acid sequence (version 2)
METDTLLLWVLLLWVPGSTGEVQLQQSGPELIKPGASVKMSCKASGYTFTSYVMHWVKQKPGQGLEWIGYINPYNDGTKYNEKFKGKATLTSDKSSSTAYMELSSLTSEDSAVYYCARGTYYYGSRVFDYWGQGTTLTVSSGGGGSGGGGSGGGGSDIVMTQAAPSIPVTPGESVSISCRSSKSLLNSNGNTYLYWFLQRPGQSPQLLIYRMSNLASGVPDRFSGSGSGTAFTLRISRVEAEDVGVYYCMQHLEYPFTFGAGTKLELKRSDPTTTPAPRPPTPAPTIASQPLSLRPEACRPAAGGAVHTRGLDFACDIYIWAPLAGTCGVLLLSLVITLYCKRGRKKLLYIFKQPFMRPVQTTQEEDGCSCRFPEEEEGGCELRVKFSRSADAPAYQQGQNQLYNELNLGRREEYDVLDKRRGRDPEMGGKPRRKNPQEGLYNELQKDKMAEAYSEIGMKGERRRGKGHDGLYQGLSTATKDTYDALHMQALPPR

SEQ ID NO: 2 - protein, 5 aa, Artificial Sequence
  CD52 antibody HCDR1
DFYMN

SEQ ID NO: 3 - protein, 19 aa, Artificial Sequence
  CD52 antibody HCDR2
FIRDKAKGYTTEYNPSVKG

SEQ ID NO: 4 - protein, 10 aa, Artificial Sequence
  CD52 antibody HCDR3
EGHTAAPFDY

SEQ ID NO: 5 - protein, 11 aa, Artificial Sequence
  CD52 antibody LCDR1
KASQNIDKYLN

SEQ ID NO: 6 - protein, 7 aa, Artificial Sequence
  CD52 antibody LCDR2
NTNNLQT

SEQ ID NO: 7 - protein, 9 aa, Artificial Sequence
  CD52 antibody LCDR3
LQHISRPRT

SEQ ID NO: 8 - protein, 451 aa, Artificial Sequence
  CD52 antibody VH
QVQLQESGPGLVRPSQTLSLTCTVSGFTFTDFYMNWVRQPPGRGLEWIGFIRDKAKGYTTEYNPSVKGRVTMLVDTSKNQFSLRLSSVTAADTAVYYCAREGHTAAPFDYWGQGSLVTVSSASTKGPSVFPLAPSSKSTSGGTAALGCLVKDYFPEPVTVSWNSGALTSGVHTFPAVLQSSGLYSLSSVVTVPSSSLGTQTYICNVNHKPSNTKVDKKVEPKSCDKTHTCPPCPAPELLGGPSVFLFPPKPKDTLMISRTPEVTCVVVDVSHEDPEVKFNWYVDGVEVHNAKTKPREEQYNSTYRVVSVLTVLHQDWLNGKEYKCKVSNKALPAPIEKTISKAKGQPREPQVYTLPPSRDELTKNQVSLTCLVKGFYPSDIAVEWESNGQPENNYKTTPPVLDSDGSFFLYSKLTVDKSRWQQGNVFSCSVMHEALHNHYTQKSLSLSPGK

SEQ ID NO: 9 - DNA, 1353 bp, Artificial Sequence
  CD52 antibody VH
caagtgcagcttcaagaatccggccctggtctggtccgcccctcccaaaccctctccctgacatgcaccgtgtcgggattcacctttaccgatttctacatgaactgggtccggcagccgcccggaagaggtctggagtggatcggcttcattcgggacaaagccaaggggtacaccaccgagtacaacccgtccgtgaagggacgcgtgactatgctcgtggacacgtccaagaaccagttcagcttgaggctgagcagcgtgactgccgcggataccgcagtgtactactgtgcccgggaagggcacactgccgctccattcgactattggggccagggatcactggtcactgtgtcgtccgcctccaccaagggcccatcggtcttccccctggcaccctcctccaagagcacctctgggggcacagcggccctgggctgcctggtcaaggactacttccccgaaccggtgacggtgtcgtggaactcaggcgccctgaccagcggcgtgcacaccttcccggctgtcctacagtcctcaggactctactccctcagcagcgtagtgaccgtgccctccagcagcttgggcacccagacctacatctgcaacgtgaatcacaagcccagcaacaccaaggtggacaagaaagttgagcccaaatcttgtgacaaaactcacacatgcccaccgtgcccagcacctgaactcctggggggaccgtcagtcttcctcttccccccaaaacccaaggacaccctcatgatctcccggacccctgaggtcacatgcgtggtggtggacgtgagccacgaagaccctgaggtcaagttcaactggtacgtggacggcgtggaggtgcataatgccaagacaaagccgcgggaggagcagtacaacagcacgtaccgtgtggtcagcgtcctcaccgtcctgcaccaggactggctgaatggcaaggagtacaagtgcaaggtctccaacaaagccctcccagcccccatcgagaaaaccatctccaaagccaaagggcagccccgagaaccacaggtgtacaccctgcccccatcccgggacgagctgaccaagaaccaggtcagcctgacctgcctggtcaaaggcttctatcccagcgacatcgccgtggagtgggagagcaatgggcagccggagaacaactacaagaccacgcctcccgtgctggactccgacggctccttcttcctctatagcaagctcaccgtggacaagagcaggtggcagcaggggaacgtcttctcatgctccgtgatgcatgaggctctgcacaaccactacacgcagaagagcctctccctgtctccgggaaaa

SEQ ID NO: 10 - protein, 214 aa, Artificial Sequence
  CD52 antibody VL
DIQMTQSPSSLSASVGDRVTITCKASQNIDKYLNWYQQKPGKAPKLLIYNTNNLQTGVPSRFSGSGSGTDFTFTISSLQPEDIATYYCLQHISRPRTFGQGTKVEIKRTVAAPSVFIFPPSDEQLKSGTASVVCLLNNFYPREAKVQWKVDNALQSGNSQESVTEQDSKDSTYSLSSTLTLSKADYEKHKVYACEVTHQGLSSPVTKSFNRGEC

SEQ ID NO: 11 - DNA, 699 bp, Artificial Sequence
  CD52 antibody VL
atgggatggagctgtatcatcctcttcttggtagcaacagctacaggcgtgcactccgacatccaaatgacccaatccccatcctcactttccgcctccgtgggcgaccgcgtgactattacctgtaaagcgtcacagaatatcgacaagtacctgaactggtaccagcagaagcctggaaaggcccccaagctcctgatctacaacaccaacaacttgcagactggagtgccgagcagattttccggctccggctcggggactgatttcaccttcaccatctcgagcctgcagccggaggatattgctacctattactgcctgcaacacattagccggcccaggacgttcggacagggtaccaaggtcgaaatcaagcgtacggtggctgcaccatctgtcttcatcttcccgccatctgatgagcagttgaaatctggaactgcctctgttgtgtgcctgctgaataacttctatcccagagaggccaaagtacagtggaaggtggataacgccctccaatcgggtaactcccaggagagtgtcacagagcaggacagcaaggacagcacctacagcctcagcagcaccctgacgctgagcaaagcagactacgagaaacacaaagtctacgcctgcgaagtcacccatcagggcctgagctcgcccgtcacaaagagcttcaacaggggagagtgt

SEQ ID NO: 12 - protein, 177 aa, Artificial Sequence
  Full length RQR8 safety switch
MLTSLLCWMALCLLGADHADACPYSNPSLCSGGGGSELPTQGTFSNVSTNVSPAKPTTTACPYSNPSLCSGGGGSPAPRPPTPAPTIASQPLSLRPEACRPAAGGAVHTRGLDFACDIYIWAPLAGTCGVLLLSLVITLYCNHRNRRRVCKCPRPVVRAEGRGSLLTCGDVEENPGP

SEQ ID NO: 13 - protein, 21 aa, Artificial Sequence
  Human TCR beta leader sequence (with G to L substitution)
MLTSLLCWMALCLLGADHADA

SEQ ID NO: 14 - protein, 9 aa, Artificial Sequence
  Rituximab epitope
CPYSNPSLC

SEQ ID NO: 15 - protein, 6 aa, Artificial Sequence
  glycine-serine linker
SGGGGS

SEQ ID NO: 16 - protein, 16 aa, Homo sapiens
ELPTQGTFSNVSTNVS

SEQ ID NO: 17 - protein, 7 aa, Homo sapiens
PAKPTTT

SEQ ID NO: 18 - protein, 42 aa, Homo sapiens
PAPRPPTPAPTIASQPLSLRPEACRPAAGGAVHTRGLDFACD

SEQ ID NO: 19 - protein, 21 aa, Homo sapiens
IYIWAPLAGTCGVLLLSLVIT

SEQ ID NO: 20 - protein, 19 aa, Homo sapiens
LYCNHRNRRRVCKCPRPVV

SEQ ID NO: 21 - protein, 19 aa, Thosea asigna virus
RAEGRGSLLTCGDVEENPG

SEQ ID NO: 22 - protein, 495 aa, Artificial Sequence
  CAR full length amino acid sequence (version 1)
MALPVTALLLPLALLLHAARPEVQLQQSGPELIKPGASVKMSCKASGYTFTSYVMHWVKQKPGQGLEWIGYINPYNDGTKYNEKFKGKATLTSDKSSSTAYMELSSLTSEDSAVYYCARGTYYYGSRVFDYWGQGTTLTVSSGGGGSGGGGSGGGGSDIVMTQAAPSIPVTPGESVSISCRSSKSLLNSNGNTYLYWFLQRPGQSPQLLIYRMSNLASGVPDRFSGSGSGTAFTLRISRVEAEDVGVYYCMQHLEYPFTFGAGTKLELKRADTTTPAPRPPTPAPTIASQPLSLRPEACRPAAGGAVHTRGLDFACDIYIWAPLAGTCGVLLLSLVITLYCKRGRKKLLYIFKQPFMRPVQTTQEEDGCSCRFPEEEEGGCELRVKFSRSADAPAYQQGQNQLYNELNLGRREEYDVLDKRRGRDPEMGGKPRRKNPQEGLYNELQKDKMAEAYSEIGMKGERRRGKGHDGLYQGLSTATKDTYDALHMQALPPR

SEQ ID NO: 23 - protein, 672 aa, Artificial Sequence
  UCART19 CAR full length amino acid sequence with RQR8 safety switch
MLTSLLCWMALCLLGADHADACPYSNPSLCSGGGGSELPTQGTFSNVSTNVSPAKPTTTACPYSNPSLCSGGGGSPAPRPPTPAPTIASQPLSLRPEACRPAAGGAVHTRGLDFACDIYIWAPLAGTCGVLLLSLVITLYCNHRNRRRVCKCPRPVVRAEGRGSLLTCGDVEENPGPMETDTLLLWVLLLWVPGSTGEVQLQQSGPELIKPGASVKMSCKASGYTFTSYVMHWVKQKPGQGLEWIGYINPYNDGTKYNEKFKGKATLTSDKSSSTAYMELSSLTSEDSAVYYCARGTYYYGSRVFDYWGQGTTLTVSSGGGGSGGGGSGGGGSDIVMTQAAPSIPVTPGESVSISCRSSKSLLNSNGNTYLYWFLQRPGQSPQLLIYRMSNLASGVPDRFSGSGSGTAFTLRISRVEAEDVGVYYCMQHLEYPFTFGAGTKLELKRSDPTTTPAPRPPTPAPTIASQPLSLRPEACRPAAGGAVHTRGLDFACDIYIWAPLAGTCGVLLLSLVITLYCKRGRKKLLYIFKQPFMRPVQTTQEEDGCSCRFPEEEEGGCELRVKFSRSADAPAYQQGQNQLYNELNLGRREEYDVLDKRRGRDPEMGGKPRRKNPQEGLYNELQKDKMAEAYSEIGMKGERRRGKGHDGLYQGLSTATKDTYDALHMQALPPR

SEQ ID NO: 24 - protein, 20 aa, Mus musculus
METDTLLLWVLLLWVPGSTG

SEQ ID NO: 25 - protein, 121 aa, Mus musculus
EVQLQQSGPELIKPGASVKMSCKASGYTFTSYVMHWVKQKPGQGLEWIGYINPYNDGTKYNEKFKGKATLTSDKSSSTAYMELSSLTSEDSAVYYCARGTYYYGSRVFDYWGQGTTLTVSS

SEQ ID NO: 26 - protein, 15 aa, Artificial Sequence
  Glycine-serine linker
GGGGSGGGGSGGGGS

SEQ ID NO: 27 - protein, 115 aa, Artificial Sequence
  Mouse anti-human CD19 (4G7) kappa light chain (with A to S substitution) (CDRs)
DIVMTQAAPSIPVTPGESVSISCRSSKSLLNSNGNTYLYWFLQRPGQSPQLLIYRMSNLASGVPDRFSGSGSGTAFTLRISRVEAEDVGVYYCMQHLEYPFTFGAGTKLELKRSD

SEQ ID NO: 28 - protein, 252 aa, Artificial Sequence
  Extracellular binding domain (version 2)
EVQLQQSGPELIKPGASVKMSCKASGYTFTSYVMHWVKQKPGQGLEWIGYINPYNDGTKYNEKFKGKATLTSDKSSSTAYMELSSLTSEDSAVYYCARGTYYYGSRVFDYWGQGTTLTVSSGGGGSGGGGSGGGGSDIVMTQAAPSIPVTPGESVSISCRSSKSLLNSNGNTYLYWFLQRPGQSPQLLIYRMSNLASGVPDRFSGSGSGTAFTLRISRVEAEDVGVYYCMQHLEYPFTFGAGTKLELKRSDP

SEQ ID NO: 29 - protein, 251 aa, Artificial Sequence
  Extracellular binding domain (version 1)
EVQLQQSGPELIKPGASVKMSCKASGYTFTSYVMHWVKQKPGQGLEWIGYINPYNDGTKYNEKFKGKATLTSDKSSSTAYMELSSLTSEDSAVYYCARGTYYYGSRVFDYWGQGTTLTVSSGGGGSGGGGSGGGGSDIVMTQAAPSIPVTPGESVSISCRSSKSLLNSNGNTYLYWFLQRPGQSPQLLIYRMSNLASGVPDRFSGSGSGTAFTLRISRVEAEDVGVYYCMQHLEYPFTFGAGTKLELKRAD

SEQ ID NO: 30 - protein, 46 aa, Homo sapiens
PTTTPAPRPPTPAPTIASQPLSLRPEACRPAAGGAVHTRGLDFACD

SEQ ID NO: 31 - protein, 21 aa, Homo sapiens
IYIWAPLAGTCGVLLLSLVIT

SEQ ID NO: 32 - protein, 69 aa, Artificial Sequence
  Fragment of T-cell surface glycoprotein CD8 alpha chain isoform 1 precursor (residues 138-206)
TTTPAPRPPTPAPTIASQPLSLRPEACRPAAGGAVHTRGLDFACDIYIWAPLAGTCGVLLLSLVITLYC

SEQ ID NO: 33 - protein, 3 aa, Homo sapiens
LYC

SEQ ID NO: 34 - protein, 42 aa, Homo sapiens
KRGRKKLLYIFKQPFMRPVQTTQEEDGCSCRFPEEEEGGCEL

SEQ ID NO: 35 - protein, 112 aa, Homo sapiens
RVKFSRSADAPAYQQGQNQLYNELNLGRREEYDVLDKRRGRDPEMGGKPRRKNPQEGLYNELQKDKMAEAYSEIGMKGERRRGKGHDGLYQGLSTATKDTYDALHMQALPPR